European Patent Application EP 4 697 024 A2, published February 18, 2026. Title: DIAGNOSTIC AND PROGNOSTIC BIOMARKER PROFILES IN PATIENTS WITH HEMATOPOIETIC STEM CELL TRANSPLANT-ASSOCIATED THROMBOTIC MICROANGIOPATHY (HSCT-TMA). Applicant: ALEXION PHARMACEUTICALS, INC. The sequence listing filed with the application follows.

SEQUENCE LISTING (51 sequences)

SEQ ID NO: 1 - protein, 10 aa, synthetic construct
GYIFSNYWIQ

SEQ ID NO: 2 - protein, 17 aa, synthetic construct
EILPGSGSTEYTENFKD

SEQ ID NO: 3 - protein, 13 aa, synthetic construct
YFFGSSPNWYFDV

SEQ ID NO: 4 - protein, 11 aa, synthetic construct
GASENIYGALN

SEQ ID NO: 5 - protein, 7 aa, synthetic construct
GATNLAD

SEQ ID NO: 6 - protein, 9 aa, synthetic construct
QNVLNTPLT

SEQ ID NO: 7 - protein, 122 aa, synthetic construct [sequence omitted]

SEQ ID NO: 8 - protein, 107 aa, synthetic construct [sequence omitted]

SEQ ID NO: 9 - protein, 326 aa, synthetic construct
ASTKGPSVFPLAPCSRSTSESTAALGCLVKDYFPEPVTVSWNSGALTSGVHTFPAVLQSSGLYSLSSVVTVPSSNFGTQTYTCNVDHKPSNTKVDKTVERKCCVECPPCPAPPVAGPSVFLFPPKPKDTLMISRTPEVTCVVVDVSQEDPEVQFNWYVDGVEVHNAKTKPREEQFNSTYRVVSVLTVLHQDWLNGKEYKCKVSNKGLPSSIEKTISKAKGQPREPQVYTLPPSQEEMTKNQVSLTCLVKGFYPSDIAVEWESNGQPENNYKTTPPVLDSDGSFFLYSRLTVDKSRWQEGNVFSCSVMHEALHNHYTQKSLSLSLGK

SEQ ID NO: 10 - protein, 447 aa, synthetic construct
QVQLVQSGAEVKKPGASVKVSCKASGYIFSNYWIQWVRQAPGQGLEWMGEILPGSGSTEYTENFKDRVTMTRDTSTSTVYMELSSLRSEDTAVYYCARYFFGSSPNWYFDVWGQGTLVTVSSASTKGPSVFPLAPCSRSTSESTAALGCLVKDYFPEPVTVSWNSGALTSGVHTFPAVLQSSGLYSLSSVVTVPSSNFGTQTYTCNVDHKPSNTKVDKTVERKCCVECPPCPAPPVAGPSVFLFPPKPKDTLMISRTPEVTCVVVDVSQEDPEVQFNWYVDGVEVHNAKTKPREEQFNSTYRVVSVLTVLHQDWLNGKEYKCKVSNKGLPSSIEKTISKAKGQPREPQVYTLPPSQEEMTNQVSLTCLVKGFYPSDIAVEWESNGQPENNYKTTPPVLDSDGSFFLYSRLTVDKSRWQEGNVFSCSVMHEALHNHYTQKSLSLSLGK

SEQ ID NO: 11 - protein, 214 aa, synthetic construct [sequence omitted]

SEQ ID NO: 12 - protein, 122 aa, synthetic construct [sequence omitted]

SEQ ID NO: 13 - protein, 326 aa, synthetic construct
ASTKGPSVFPLAPCSRSTSESTAALGCLVKDYFPEPVTVSWNSGALTSGVHTFPAVLQSSGLYSLSSVVTVPSSNFGTQTYTCNVDHKPSNTKVDKTVERKCCVECPPCPAPPVAGPSVFLFPPKPKDTLMISRTPEVTCVVVDVSQEDPEVQFNWYVDGVEVHNAKTKPREEQFNSTYRVVSVLTVLHQDWLNGKEYKCKVSNKGLPSSIEKTISKAKGQPREPQVYTLPPSQEEMTKNQVSLTCLVKGFYPSDIAVEWESNGQPENNYKTTPPVLDSDGSFFLYSRLTVDKSRWQEGNVFSCSVLHEALHSHYTQKSLSLSLGK

SEQ ID NO: 14 - protein, 448 aa, synthetic construct
QVQLVQSGAEVKKPGASVKVSCKASGHIFSNYWIQWVRQAPGQGLEWMGEILPGSGHTEYTENFKDRVTMTRDTSTSTVYMELSSLRSEDTAVYYCARYFFGSSPNWYFDVWGQGTLVTVSSASTKGPSVFPLAPCSRSTSESTAALGCLVKDYFPEPVTVSWNSGALTSGVHTFPAVLQSSGLYSLSSVVTVPSSNFGTQTYTCNVDHKPSNTKVDKTVERKCCVECPPCPAPPVAGPSVFLFPPKPKDTLMISRTPEVTCVVVDVSQEDPEVQFNWYVDGVEVHNAKTKPREEQFNSTYRVVSVLTVLHQDWLNGKEYKCKVSNKGLPSSIEKTISKAKGQPREPQVYTLPPSQEEMTKNQVSLTCLVKGFYPSDIAVEWESNGQPENNYKTTPPVLDSDGSFFLYSRLTVDKSRWQEGNVFSCSVLHEALHSHYTQKSLSLSLGK

SEQ ID NO: 15 - protein, 326 aa, synthetic construct
ASTKGPSVFPLAPCSRSTSESTAALGCLVKDYFPEPVTVSWNSGALTSGVHTFPAVLQSSGLYSLSSVVTVTSSNFGTQTYTCNVDHKPSNTKVDKTVERKCCVECPPCPAPPVAGPSVFLFPPKPKDTLYITREPEVTCVVVDVSHEDPEVQFNWYVDGMEVHNAKTKPREEQFNSTFRVVSVLTVVHQDWLNGKEYKCKVSNKGLPAPIEKTISKTKGQPREPQVYTLPPSREEMTKNQVSLTCLVKGFYPSDIAVEWESNGQPENNYKTTPPMLDSDGSFFLYSKLTVDKSRWQQGNVFSCSVMHEALHNHYTQKSLSLSPGK

SEQ ID NO: 16 - protein, 448 aa, synthetic construct
QVQLVQSGAEVKKPGASVKVSCKASGYIFSNYWIQWVRQAPGQGLEWMGEILPGSGSTEYTENFKDRVTMTRDTSTSTVYMELSSLRSEDTAVYYCARYFFGSSPNWYFDVWGQGTLVTVSSASTKGPSVFPLAPCSRSTSESTAALGCLVKDYFPEPVTVSWNSGALTSGVHTFPAVLQSSGLYSLSSVVTVTSSNFGTQTYTCNVDHKPSNTKVDKTVERKCCVECPPCPAPPVAGPSVFLFPPKPKDTLYITREPEVTCVVVDVSHEDPEVQFNWYVDGMEVHNAKTKPREEQFNSTFRVVSVLTVVHQDWLNGKEYKCKVSNKGLPAPIEKTISKTKGQPREPQVYTLPPSREEMTKNQVSLTCLVKGFYPSDIAVEWESNGQPENNYKTTPPMLDSDGSFFLYSKLTVDKSRWQQGNVFSCSVMHEALHNHYTQKSLSLSPGK

SEQ ID NO: 17 - protein, 11 aa, synthetic construct
GASENIYHALN

SEQ ID NO: 18 - protein, 17 aa, synthetic construct
EILPGSGHTEYTENFKD

SEQ ID NO: 19 - protein, 10 aa, synthetic construct
GHIFSNYWIQ

SEQ ID NO: 20 - protein, 448 aa, synthetic construct
QVQLVQSGAEVKKPGASVKVSCKASGHIFSNYWIQWVRQAPGQGLEWMGEILPGSGHTEYTENFKDRVTMTRDTSTSTVYMELSSLRSEDTAVYYCARYFFGSSPNWYFDVWGQGTLVTVSSASTKGPSVFPLAPCSRSTSESTAALGCLVKDYFPEPVTVSWNSGALTSGVHTFPAVLQSSGLYSLSSVVTVPSSNFGTQTYTCNVDHKPSNTKVDKTVERKCCVECPPCPAPPVAGPSVFLFPPKPKDTLMISRTPEVTCVVVDVSQEDPEVQFNWYVDGVEVHNAKTKPREEQFNSTYRVVSVLTVLHQDWLNGKEYKCKVSNKGLPSSIEKTISKAKGQPREPQVYTLPPSQEEMTKNQVSLTCLVKGFYPSDIAVEWESNGQPENNYKTTPPVLDSDGSFFLYSRLTVDKSRWQEGNVFSCSVMHEALHNHYTQKSLSLSLGK

SEQ ID NO: 21 - protein, 5 aa, synthetic construct
SYAIS

SEQ ID NO: 22 - protein, 17 aa, synthetic construct
GIGPFFGTANYAQKFQG

SEQ ID NO: 23 - protein, 7 aa, synthetic construct
DTPYFDY

SEQ ID NO: 24 - protein, 11 aa, synthetic construct
SGDSIPNYYVY

SEQ ID NO: 25 - protein, 7 aa, synthetic construct
DDSNRPS

SEQ ID NO: 26 - protein, 11 aa, synthetic construct
QSFDSSLNAEV

SEQ ID NO: 27 - protein, 116 aa, synthetic construct
QVQLVQSGAEVKKPGSSVKVSCKASGGTFSSYAISVWRQAPGQGLEWMGGIGPFFGTANYAQKFQGRVTITADESTSTAYMELSSLRSEDTAVYYCARDTPYFDYWGQGTLVTVSS

SEQ ID NO: 28 - protein, 108 aa, synthetic construct
DIELTQPPSVSVAPGQTARISCSGDSIPNYYVYWYQQKPGQAPVLVIYDDSNRPSGIPERFSGSNSGNTATLTISGTQAEDEADYYCQSFDSSLNAEVFGGGTKLTVL

SEQ ID NO: 29 - protein, 4 aa, synthetic construct
NYIS

SEQ ID NO: 30 - protein, 17 aa, synthetic construct
IIDPDDSYTEYSPSFQG

SEQ ID NO: 31 - protein, 8 aa, synthetic construct
YEYGGFDI

SEQ ID NO: 32 - protein, 11 aa, synthetic construct
SGDNIGNSYVH

SEQ ID NO: 33 - protein, 7 aa, synthetic construct
KDNDRPS

SEQ ID NO: 34 - protein, 9 aa, synthetic construct
GTYDIESYV

SEQ ID NO: 35 - protein, 116 aa, synthetic construct
EVQLVQSGAEVKKPGESLKISCKGSGYSFTNYISWVRQMPGKGLEWMGIIDPDDSYTEYSPSFQGQVTISADKSISTAYLQWSSLKASDTAMYYCARYEYGGFDIWGQGTLVTVSS

SEQ ID NO: 36 - protein, 106 aa, synthetic construct
SYELTQPPSVSVAPGQTARISCSGDNIGNSYVHWYQQKPGQAPVLVIYKDNDRPSGIPERFSGSNSGNTATLTISGTQAEDEADYYCGTYDIESYVFGGGTKLTVL

SEQ ID NO: 37 - protein, 6 aa, synthetic construct
SSYYVA

SEQ ID NO: 38 - protein, 17 aa, synthetic construct
AIYTGSGATYKASWAKG

SEQ ID NO: 39 - protein, 13 aa, synthetic construct
DGGYDYPTHAMHY

SEQ ID NO: 40 - protein, 11 aa, synthetic construct
QASQNIGSSLA

SEQ ID NO: 41 - protein, 7 aa, synthetic construct
GASKTHS

SEQ ID NO: 42 - protein, 12 aa, synthetic construct
QSTKVGSSYGNH

SEQ ID NO: 43 - protein, 123 aa, synthetic construct
QVQLVESGGGLVQPGGSLRLSCAASGFTSHSSYYVAWVRQAPGKGLEWVGAIYTGSGATYKASWAKGRFTISKDTSKNQVVLTMTNMDPVDTATYYCASDGGYDYPTHAMHYWGQGTLVTVSS

SEQ ID NO: 44 - protein, 110 aa, synthetic construct
DVVMTQSPSSLSASVGDRVTITCQASQNIGSSLAWYQQKPGQAPRLLIYGASKTHSGVPSRFSGSGSGTDFTLTISSLQPEDVATYYCQSTKVGSSYGNHFGGGTKVEIK

SEQ ID NO: 45 - protein, 451 aa, synthetic construct
QVQLVESGGGLVQPGRSLRLSCAASGFTVHSSYYMAWVRQAPGKGLEWVGAIFTGSGAEYKAEWAKGRVTISKDTSKNQVVLTMTNMDPVDTATYYCASDAGYDYPTHAMHYWGQGTLVTVSSASTKGPSVFPLAPSSKSTSGGTAALGCLVKDYFPEPVTVSWNSGALTSGVHTFPAVLQSSGLYSLSSVVTVPSSSLGTQTYICNVNHKPSNTKVDKKVEPKSCDKTHTCPPCPAPELRRGPKVFLFPPKPKDTLMISRTPEVTCVVVDVSHEDPEVKFNWYVDGVEVHNAKTKPREEQYNSTYRVVSVLTVLHQDWLNGKEYKCKVSNKGLPSSIEKTISKAKGQPREPQVYTLPPSREEMTKNQVSLTCLVKGFYPSDIAVEWESNGQPENNYKTTPPVLDSDGSFFLYSKLTVDKSRWQQGNVFSCSVLHEALHAHYTRKELSLSP

SEQ ID NO: 46 - protein, 217 aa, synthetic construct
DIQMTQSPSSLSASVGDRVTITCRASQGISSSLAWYQQKPGKAPKLLIYGASETESGVPSRFSGSGSGTDFTLTISSLQPEDFATYYCQNTKVGSSYGNTFGGGTKVEIKRTVAAPSVFIFPPSDEQLKSGTASVVCLLNNFYPREAKVQWKVDNALQSGNSQESVTEQDSKDSTYSLSSTLTLSKADYEKHKVYACEVTHQGLSSPVTKSFNRGEC

SEQ ID NO: 47 - protein, 120 aa, synthetic construct
QVQLQESGPGLVKPSETLSLTCTVSGDSVSSSYWTWIRQPPGKGLEWIGYIYYSGSSNYNPSLKSRATISVDTSKNQFSLKLSSVTAADTAVYYCAREGNVDTTMIFDYWGQGTLVTVSS

SEQ ID NO: 48 - protein, 107 aa, synthetic construct
AIQMTQSPSSLSASVGDRVTITCRASQGIRNDLGWYQQKPGKAPKLLIYAASSLQSGVPSRFAGRGSGTDFTLTISSLQPEDFATYYCLQDFNYPWTFGQGTKVEIK

SEQ ID NO: 49 - protein, 447 aa, synthetic construct
QVQLQESGPGLVKPSETLSLTCTVSGDSVSSSYWTWIRQPPGKGLEWIGYIYYSGSSNYNPSLKSRATISVDTSKNQFSLKLSSVTAADTAVYYCAREGNVDTTMIFDYWGQGTLVTVSSASTKGPSVFPLAPCSRSTSESTAALGCLVKDYFPEPVTVSWNSGALTSGVHTFPAVLQSSGLYSLSSVVTVPSSSLGTKTYTCNVDHKPSNTKVDKRVESKYGPPCPPCPAPEFLGGPSVFLFPPKPKDTLMISRTPEVTCVVVDVSQEDPEVQFNWYVDGVEVHNAKTKPREEQFNSTYRVVSVLTVLHQDWLNGKEYKCKVSNKGLPSSIEKTISKAKGQPREPQVYTLPPSQEEMTKNQVSLTCLVKGFYPSDIAVEWESNGQPENNYKTTPPVLDSDGSFFLYSRLTVDKSRWQEGNVFSCSVMHEALHNHYTQKSLSLSLGK

SEQ ID NO: 50 - protein, 214 aa, synthetic construct
AIQMTQSPSSLSASVGDRVTITCRASQGIRNDLGWYQQKPGKAPKLLIYAASSLQSGVPSRFAGRGSGTDFTLTISSLQPEDFATYYCLQDFNYPWTFGQGTKVEIKRTVAAPSVFIFPPSDEQLKSGTASVVCLLNNFYPREAKVQWKVDNALQSGNSQESVTEQDSKDSTYSLSSTLTLSKADYEKHKVYACEVTHQGLSSPVTKSFNRGEC

SEQ ID NO: 51 - protein, 6 aa, synthetic construct
HHHHHH